European Patent Application EP 4 382 603 A1, published June 12, 2024. Title: Artificial oligonucleotides which induces specific 3-dimentional structure. Applicant: Sophia School Corporation. The sequence listing filed with the application follows.

SEQUENCE LISTING (44 sequences)

SEQ ID NO: 1-12 - skipped (12 entries)

SEQ ID NO: 13 - RNA, 26 nt, synthetic construct
  misc_feature 1..26: note = synthetic
  source 1..26: mol_type = other RNA
catggctcttgcagatgcgatgttgc

SEQ ID NO: 14 - RNA, 27 nt, synthetic construct
  misc_feature 1..27: note = synthetic
  source 1..27: mol_type = other RNA
gcaacatcgtagtatgcaagagccatg

SEQ ID NO: 15 - RNA, 29 nt, synthetic construct
  misc_feature 1..29: note = synthetic
  source 1..29: mol_type = other RNA
gcaacatcgcagaagatgcaagagccatg

SEQ ID NO: 16 - RNA, 29 nt, synthetic construct
  misc_feature 1..29: note = synthetic
  source 1..29: mol_type = other RNA
gcaacatcgcaacaaatgcaagagccatg

SEQ ID NO: 17 - RNA, 26 nt, synthetic construct
  misc_feature 1..26: note = synthetic
  source 1..26: mol_type = other RNA
gcaacatcgcgtatgcaagagccatg

SEQ ID NO: 18 - RNA, 28 nt, synthetic construct
  misc_feature 1..28: note = synthetic
  source 1..28: mol_type = other RNA
gcaacatcgccactctgcaagagccatg

SEQ ID NO: 19 - RNA, 26 nt, synthetic construct
  misc_feature 1..26: note = synthetic
  source 1..26: mol_type = other RNA
gcaacatcgcagatgcaagagccatg

SEQ ID NO: 20 - RNA, 26 nt, synthetic construct
  misc_feature 1..26: note = synthetic
  source 1..26: mol_type = other RNA
gcaacatcgcatctgcaagagccatg

SEQ ID NO: 21 - RNA, 27 nt, synthetic construct
  misc_feature 1..27: note = synthetic
  misc_feature 1..27: note = 5'-O-Me RNA
  source 1..27: mol_type = other RNA
gcaacatcgtagtatgcaagagccatg

SEQ ID NO: 22 - RNA, 26 nt, synthetic construct
  misc_feature 1..26: note = synthetic
  misc_feature 1..26: note = 5'-O-Me RNA
  source 1..26: mol_type = other RNA
gcaacatcgcgtatgcaagagccatg

SEQ ID NO: 23 - RNA, 26 nt, synthetic construct
  misc_feature 1..26: note = synthetic
  misc_feature 1..26: note = 5'-O-Me RNA
  source 1..26: mol_type = other RNA
gcaacatcgcagatgcaagagccatg

SEQ ID NO: 24 - RNA, 26 nt, synthetic construct
  misc_feature 1..26: note = synthetic
  misc_feature 1..26: note = 5'-O-Me RNA
  source 1..26: mol_type = other RNA
gcaacatcgcatctgcaagagccatg

SEQ ID NO: 25 - RNA, 27 nt, synthetic construct
  misc_feature 1..27: note = synthetic
  source 1..27: mol_type = other RNA
tgctcctagtacgagaggaccggagtg

SEQ ID NO: 26 - DNA, 27 bp, synthetic construct
  misc_feature 1..27: note = synthetic
  misc_feature order(1..7, 10..12): note = 5'-O-Me RNA
  misc_feature 13..27: note = RNA
  misc_feature 1..12: note = DNA
  source 1..27: mol_type = other DNA
tgctcctagtacgagaggaccggagtg

SEQ ID NO: 27 - RNA, 19 nt, synthetic construct
  misc_feature 1..19: note = synthetic
  source 1..19: mol_type = other RNA
ggcgaagaaccggggagcc

SEQ ID NO: 28 - DNA, 19 bp, synthetic construct
  misc_feature 1..19: note = synthetic
  misc_feature order(1..11,17): note = RNA
  misc_feature order(12..16,18..19): note = DNA
  misc_feature order(12..14,18..19): note = 5'-O-Me RNA
  source 1..19: mol_type = other DNA
ggcgaagaaccggggagcc

SEQ ID NO: 29 - RNA, 35 nt, synthetic construct
  misc_feature 1..35: note = synthetic
  source 1..35: mol_type = other RNA
ctgctggctaaggcatgaaagtgctatgcctgctg

SEQ ID NO: 30 - DNA, 35 bp, synthetic construct
  misc_feature 1..35: note = synthetic
  misc_feature 1..20: note = RNA
  misc_feature 21..35: note = DNA
  source 1..35: mol_type = other DNA
cagcaggctaaggcatgaaagtgctatgcctgctg

SEQ ID NO: 31 - RNA, 19 nt, synthetic construct
  misc_feature 1..19: note = synthetic
  source 1..19: mol_type = other RNA
gggccggctttgaaccggg

SEQ ID NO: 32 - RNA, 19 nt, synthetic construct
  misc_feature 1..19: note = synthetic
  source 1..19: mol_type = other RNA
gggccggcaaagaaccggg

SEQ ID NO: 33 - RNA, 19 nt, synthetic construct
  misc_feature 1..19: note = synthetic
  source 1..19: mol_type = other RNA
cccggttcaaagccggccc

SEQ ID NO: 34 - RNA, 16 nt, synthetic construct
  misc_feature 1..16: note = synthetic
  source 1..16: mol_type = other RNA
cccggggagccggccc

SEQ ID NO: 35 - DNA, 3236 bp, synthetic construct
  misc_feature 1..3236: note = synthetic
  source 1..3236: mol_type = other DNA
agcggataacaatttcacacaggaaacagctatgaccatgattacgaattcagatctcgatcccgcgaaattaatacgactcactatagggagaccacaacggtttccctctagaaataattttgtttaactttaagaaggagatatacatatgaaagatcatctcatccacaatcatcacaaagaggagcacgctcatgcccacaacaaggattacgatatcccaactactcatcacgctcatcacagtactgagaacctgtacttccagggatccagcggctcctcgggaatgtcgaaaggcgaagaactgtttactggtgtagttccgattctggtggagttagacggtgacgttaacggtcacaaattcagtgtttccggtgaaggtgaaggagacgctacttacggtaagttaaccctgaaattcatctgtacaaccggtaaactgccggtaccttggcctacgctggtgactaccctgacttacggtgtacagtgctttagccgttatcccgatcacatgaaacgtcacgacttctttaaatctgctatgccagaaggttacgtgcaggaacgtaccatttcgtttaaagacgacggtaactacaaaacccgtgcagaagtcaaattcgaaggtgatactctggtgaatcggattgaactcaaagggatcgactttaaggaggacggtaatattctgggccataaactcgagtacaactacaacagccacaacgtgtatatcaccgcggataagcagaagaacggcatcaaagcgaacttcaaaattcgccataacatcgaagacggttctgtccaacttgccgatcattaccagcagaatacaccgattggtgacggacctgttttgcttccggacaaccattacctgtctacgcaatcagccttgtccaaagacccgaacgaaaaacgcgaccacatggtcttactggagtttgttacggcagctggcattacgcacggtatggacgagctgtataaatcggggccctcgtcaggataataatccggtaccccgcccacggctgctaacaaagcccgaaaggaagctgagttggctgctgccaccgctgagcaataactagcataaccccttggggcctctaaacgggtcttgaggggttttttgctgaaaggaggaactatatccggataacctcgagctgcaggcatgcaagcttggcactggccgtcgttttacaacgtcgtgactgggaaaaccctggcgctgcattaatgaatcggccaacgcgcggggagaggcggtttgcgtattgggcgctcttccgcttcctcgctcactgactcgctgcgctcggtcgttcggctgcggcgagcggtatcagctcactcaaaggcggtaatacggttatccacagaatcaggggataacgcaggaaagaacatgtgagcaaaaggccagcaaaaggccaggaaccgtaaaaaggccgcgttgctggcgtttttccataggctccgcccccctgacgagcatcacaaaaatcgacgctcaagtcagaggtggcgaaacccgacaggactataaagataccaggcgtttccccctggaagctccctcgtgcgctctcctgttccgaccctgccgcttaccggatacctgtccgcctttctcccttcgggaagcgtggcgctttctcatagctcacgctgtaggtatctcagttcggtgtaggtcgttcgctccaagctgggctgtgtgcacgaaccccccgttcagcccgaccgctgcgccttatccggtaactatcgtcttgagtccaacccggtaagacacgacttatcgccactggcagcagccactggtaacaggattagcagagcgaggtatgtaggcggtgctacagagttcttgaagtggtggcctaactacggctacactagaagaacagtatttggtatctgcgctctgctgaagccagttaccttcggaaaaagagttggtagctcttgatccggcaaacaaaccaccgctggtagcggtggtttttttgtttgcaagcagcagattacgcgcagaaaaaaaggatctcaagaagatcctttgatcttttctacggggtctgacgctcagtggaacgaaaactcacgttaagggattttggtcatgagattatcaaaaaggatcttcacctagatccttttaaattaaaaatgaagttttaaatcaatctaaagtatatatgagtaaacttggtctgacagttaccaatgcttaatcagtgaggcacctatctcagcgatctgtctatttcgttcatccatagttgcctgactccccgtcgtgtagataactacgatacgggagggcttaccatctggccccagtgctgcaatgataccgcgagacccacgctcaccggctccagatttatcagcaataaaccagccagccggaagggccgagcgcagaagtggtcctgcaactttatccgcctccatccagtctattaattgttgccgggaagctagagtaagtagttcgccagttaatagtttgcgcaacgttgttgccattgctacaggcatcgtggtgtcacgctcgtcgtttggtatggcttcattcagctccggttcccaacgatcaaggcgagttacatgatcccccatgttgtgcaaaaaagcggttagctccttcggtcctccgatcgttgtcagaagtaagttggccgcagtgttatcactcatggttatggcagcactgcataattctcttactgtcatgccatccgtaagatgcttttctgtgactggtgagtactcaaccaagtcattctgagaatagtgtatgcggcgaccgagttgctcttgcccggcgtcaatacgggataataccgcgccacatagcagaactttaaaagtgctcatcattggaaaacgttcttcggggcgaaaactctcaaggatcttaccgctgttgagatccagttcgatgtaacccactcgtgcacccaactgatcttcagcatcttttactttcaccagcgtttctgggtgagcaaaaacaggaaggcaaaatgccgcaaaaaagggaataagggcgacacggaaatgttgaatactcatactcttcctttttcaatattattgaagcatttatcagggttattgtctcatgagcggatacatatttgaatgtatttagaaaaataaacaaataggggttccgcgcacatttccccgaaaagtgccac

SEQ ID NO: 36 - RNA, 25 nt, synthetic construct
  misc_feature 1..25: note = synthetic
  source 1..25: mol_type = other RNA
cagcggctcctcgggaatgtcgaaa

SEQ ID NO: 37 - RNA, 25 nt, synthetic construct
  misc_feature 1..25: note = synthetic
  source 1..25: mol_type = other RNA
tttcgacattcccgaggagccgctg

SEQ ID NO: 38 - RNA, 25 nt, synthetic construct
  misc_feature 1..25: note = synthetic
  source 1..25: mol_type = other RNA
tttcgacatgaccgaggagccgctg

SEQ ID NO: 39 - RNA, 28 nt, synthetic construct
  misc_feature 1..28: note = synthetic
  source 1..28: mol_type = other RNA
tttcgacatgaagaccgaggagccgctg

SEQ ID NO: 40 - RNA, 27 nt, synthetic construct
  misc_feature 1..27: note = synthetic
  source 1..27: mol_type = other RNA
actctcctcgactcttcatcatcatgt

SEQ ID NO: 41 - RNA, 17 nt, synthetic construct
  misc_feature 1..17: note = synthetic
  source 1..17: mol_type = other RNA
cgagcgccccaccaccc

SEQ ID NO: 42 - RNA, 16 nt, synthetic construct
  misc_feature 1..16: note = synthetic
  source 1..16: mol_type = other RNA
gggccggtcccccggg

SEQ ID NO: 43 - RNA, 19 nt, synthetic construct
  misc_feature 1..19: note = synthetic
  source 1..19: mol_type = other RNA
cccggttcttggccggccc

SEQ ID NO: 44 - RNA, 30 nt, synthetic construct
  misc_feature 1..30: note = synthetic
  misc_feature 19: note = n = 2-aminopurine
  source 1..30: mol_type = other RNA
acatgatgatgaagaggangagaggagagt